European Patent Specification EP 3 967 329 B1, published April 1, 2026. Title: ENGINEERED IMMUNE CELL TARGETING BCMA AND USE THEREOF. Applicant: GRACELL BIOTECHNOLOGIES (SHANGHAI) CO., LTD. The sequence listing filed with the application follows.

SEQUENCE LISTING (39 sequences)

SEQ ID NO: 1 - protein, 22 aa, Artificial Sequence
  GM-CSF signal peptide
MLLLVTSLLLCELPHPAFLLIP

SEQ ID NO: 2 - protein, 20 aa, Artificial Sequence
  2A peptide
GSGATNFSLLKQAGDVEENP

SEQ ID NO: 3 - protein, 112 aa, Artificial Sequence
  CD3z signaling region
RVKFSRSADAPAYKQGQNQLYNELNLGRREEYDVLDKRRGRDPEMGGKPRRKNPQEGLYNELQKDKMAEAYSEIGMKGERRRGKGHDGLYQGLSTATKDTYDALHMQALPPR

SEQ ID NO: 4 - protein, 41 aa, Artificial Sequence
  CD28 signaling region
RSKRSRLLHSDYMNMTPRRPGPTRKHYQPYAPPRDFAAYRS

SEQ ID NO: 5 - protein, 42 aa, Artificial Sequence
  41BB signaling region
KRGRKKLLYIFKQPFMRPVQTTQEEDGCSCRFPEEEEGGCEL

SEQ ID NO: 6 - protein, 27 aa, Artificial Sequence
  CD28 transmembrane region
FWVLVVVGGVLACYSLLVTVAFIIFWV

SEQ ID NO: 7 - protein, 24 aa, Artificial Sequence
  CD8 transmembrane region
IYIWAPLAGTCGVLLLSLVITLYC

SEQ ID NO: 8 - protein, 45 aa, Artificial Sequence
  CD8 hinge region
TTTPAPRPPTPAPTIASQPLSLRPEACRPAAGGAVHTRGLDFACD

SEQ ID NO: 9 - protein, 121 aa, Artificial Sequence
  S scFv heavy chain
QVQLVQSGAEVKKPGASVKLSCKASGYTFTDYYIHWVRQAPGQGLEWIGYINPNSGYTNYAQKFQGRATMTADKSINTAYVELSRLRSDDTAVYFCTRYMWERVTGFFDFWGQGTMVTVSS

SEQ ID NO: 10 - protein, 108 aa, Artificial Sequence
  S scFv light chain
DIQMTQSPSSVSASVGDRVTITCLASEDISDDLAWYQQKPGKAPKVLVYTTSSLQSGVPSRFSGSGSGTDFTLTISSLQPEDFATYFCQQTYKFPPTFGGGTKVEIKR

SEQ ID NO: 11 - protein, 120 aa, Artificial Sequence
  FMC63 scFv heavy chain
EVKLQESGPGLVAPSQSLSVTCTVSGVSLPDYGVSWIRQPPRKGLEWLGVIWGSETTYYNSALKSRLTIIKDNSKSQVFLKMNSLQTDDTAIYYCAKHYYYGGSYAMDYWGQGTSVTVSS

SEQ ID NO: 12 - protein, 107 aa, Artificial Sequence
  FMC63 scFv light chain
DIQMTQTTSSLSASLGDRVTISCRASQDISKYLNWYQQKPDGTVKLLIYHTSRLHSGVPSRFSGSGSGTDYSLTISNLEQEDIATYFCQQGNTLPYTFGGGTKLEIT

SEQ ID NO: 13 - protein, 111 aa, Artificial Sequence
  BB scFv heavy chain
DIVLTQSPPSLAMSLGKRATISCRASESVTILGSHLIHWYQQKPGQPPTLLIQLASNVQTGVPARFSGSGSRTDFTLTIDPVEEDDVAVYYCLQSRTIPRTFGGGTKLEIK

SEQ ID NO: 14 - protein, 120 aa, Artificial Sequence
  BB scFv light chain
QIQLVQSGPELKKPGETVKISCKASGYTFTDYSINWVKRAPGKGLKWMGWINTETREPAYAYDFRGRFAFSLETSASTAYLQINNLKYEDTATYFCALDYSYAMDYWGQGTSVTVSSAAA

SEQ ID NO: 15 - protein, 142 aa, Artificial Sequence
  April chain
SVLHLVPINATSKDDSDVTEVMWQPALRRGRGLQAQGYGVRIQDAGVYLLYSQVLFQDVTFTMGQVVSREGQGRQETLFRCIRSMPSHPDRAYNSCYSAGVFHLHQGDILSVIIPRARAKLNLSPHGTFLGFVKLSGGGSDP

SEQ ID NO: 16 - protein, 21 aa, Artificial Sequence
  CD8 signal peptide
MALPVTALLLPLALLLHAARP

SEQ ID NO: 17 - protein, 15 aa, Artificial Sequence
  (G4S)3 linker peptide
GGGGSGGGGSGGGGS

SEQ ID NO: 18 - protein, 25 aa, Artificial Sequence
  (G4S)5 linker peptide
GGGGSGGGGSGGGGSGGGGSGGGGS

SEQ ID NO: 19 - protein, 18 aa, Artificial Sequence
  218 linker peptide
GSTSGSGKPGSGEGSTKG

SEQ ID NO: 20 - protein, 335 aa, Artificial Sequence
  EGFRt sequence
RKVCNGIGIGEFKDSLSINATNIKHFKNCTSISGDLHILPVAFRGDSFTHTPPLDPQELDILKTVKEITGFLLIQAWPENRTDLHAFENLEIIRGRTKQHGQFSLAVVSLNITSLGLRSLKEISDGDVIISGNKNLCYANTINWKKLFGTSGQKTKIISNRGENSCKATGQVCHALCSPEGCWGPEPRDCVSCRNVSRGRECVDKCNLLEGEPREFVENSECIQCHPECLPQAMNITCTGRGPDNCIQCAHYIDGPHCVKTCPAGVMGENNTLVWKYADAGHVCHLCHPNCTYGCTGPGLEGCPTNGPKIPSIATGMVGALLLLLVVALGIGLFM

SEQ ID NO: 21 - protein, 120 aa, Artificial Sequence
  CD19 antibody heavy chain variable region
QVQLQESGPGLVKPSETLSLTCTVSGVSLPDYGVSWIRQPPGKGLEWLGVIWGSETTYYNSALKSRLTISKDTSKSQVSLKLSSVTAADTAVYYCAKHYYYGGSYAMDYWGQGTLVTVSS

SEQ ID NO: 22 - protein, 120 aa, Artificial Sequence
  CD19 antibody heavy chain variable region
QVQLQESGPGLVKPSQTLSLTCTVSGVSLPDYGVSWIRQPPGKGLEWIGVIWGSETTYYNSALKSRVTISVDTSKNQFSLKLSSVTAADTAVYYCARHYYYGGSYAMDYWGQGTTVTVSS

SEQ ID NO: 23 - protein, 120 aa, Artificial Sequence
  CD19 antibody heavy chain variable region
QVKLQESGPGLVKPSETLSLTCTVSGVSLPDYGVSWIRQPPGKGLEWIGVIWGSETTYYNSALKSRVTISKDTSKSQVFLKLSSVTAADTAVYYCAKHYYYGGSYAMDYWGQGTLVTVSS

SEQ ID NO: 24 - protein, 120 aa, Artificial Sequence
  CD19 antibody heavy chain variable region
QVKLQESGPGLVKPSETLSLTCTVSGVSLPDYGVSWIRQPPGKGLEWLGVIWGSETTYYNSALKSRLTISKDTSKSQVFLKLSSVTAADTAVYYCAKHYYYGGSYAMDYWGQGTLVTVSS

SEQ ID NO: 25 - protein, 120 aa, Artificial Sequence
  CD19 antibody heavy chain variable region
QVQLQESGPGLVKPSQTLSLTCTVSGVSLPDYGVSWIRQPPGKGLEWIGVIWGSETTYYNSALKSRVTISKDTSKNQVSLKLSSVTAADTAVYYCAKHYYYGGSYAMDYWGQGTTVTVSS

SEQ ID NO: 26 - protein, 120 aa, Artificial Sequence
  CD19 antibody heavy chain variable region
QVQLQESGPGLVKPSQTLSLTCTVSGVSLPDYGVSWIRQPPGKGLEWIGVIWGSETTYYNSALKSRLTISKDTSKNQVSLKLSSVTAADTAVYYCAKHYYYGGSYAMDYWGQGTTVTVSS

SEQ ID NO: 27 - protein, 120 aa, Artificial Sequence
  CD19 antibody heavy chain variable region
QVQLQESGPGLVKPSQTLSLTCTVSGVSLPDYGVSWIRQPPGKGLEWLGVIWGSETTYYNSALKSRLTISKDTSKNQVSLKLSSVTAADTAVYYCAKHYYYGGSYAMDYWGQGTTVTVSS

SEQ ID NO: 28 - protein, 120 aa, Artificial Sequence
  CD19 antibody heavy chain variable region
QVQLQESGPGLVKPSQTLSVTCTVSGVSLPDYGVSWIRQPPGKGLEWLGVIWGSETTYYNSALKSRLTISKDTSKNQVSLKLSSLTAADTAVYYCAKHYYYGGSYAMDYWGQGTTVTVSS

SEQ ID NO: 29 - protein, 120 aa, Artificial Sequence
  CD19 antibody heavy chain variable region
QVQLQESGPGLVKPSQTLSVTCTVSGVSLPDYGVSWIRQPPGKGLEWLGVIWGSETTYYNAALKSRLTISKDTSKNQVSLKLSSLTAADTAVYYCAKHYYYGGSYAMDYWGQGTTVTVSS

SEQ ID NO: 30 - protein, 120 aa, Artificial Sequence
  CD19 antibody heavy chain variable region
QVKLQESGPGLVKPSETLSLTCTVSGVSLPDYGVSWIRQPPGKGLEWLGVIWGSETTYYNSALKSRLTISKDTSKNQFSLKLSSVTAADTAVYYCAKHYYYGGSYAMDYWGQGTLVTVSS

SEQ ID NO: 31 - protein, 107 aa, Artificial Sequence
  CD19 antibody light chain variable region
DIQMTQSPSSLSASVGDRVTISCRASQDISKYLNWYQQKPGKAPKLLIYHTSRLHSGVPSRFSGSGSGTDYTFTISSLQPEDIATYFCQQGNTLPYTFGGGTKLEIK

SEQ ID NO: 32 - protein, 107 aa, Artificial Sequence
  CD19 antibody light chain variable region
DIQMTQSPSSLSASVGDRVTITCRASQDISKYLNWYQQKPGKAPKLLIYHTSRLHSGVPSRFSGSGSGTDFTFTISSLQPEDIATYYCQQGNTLPYTFGGGTKLEIK

SEQ ID NO: 33 - protein, 107 aa, Artificial Sequence
  CD19 antibody light chain variable region
DIQMTQSPSSLSASVGDRVTITCRASQDISKYLNWYQQKPGGAVKLLIYHTSRLHSGVPSRFSGSGSGTDYTFTISSLQPEDIATYFCQQGNTLPYTFGGGTKLEIK

SEQ ID NO: 34 - protein, 107 aa, Artificial Sequence
  CD19 antibody light chain variable region
DIQMTQSPSSLSASVGDRVTITCRASQDISKYLNWYQQKPGKAPKLLIYHTSRLHSGVPSRFSGSGSGTDYTFTISSLQPEDIATYYCQQGNTLPYTFGGGTKLEIK

SEQ ID NO: 35 - protein, 107 aa, Artificial Sequence
  CD19 antibody light chain variable region
DIQMTQSPSSLSASVGDRVTITCRASQDISKYLNWYQQKPGKAPKLLIYHTSRLHSGVPSRFSGSGSGTDYTLTISSLQPEDIATYYCQQGNTLPYTFGGGTKLEIK

SEQ ID NO: 36 - protein, 107 aa, Artificial Sequence
  CD19 antibody light chain variable region
DIQMTQSPSSLSASVGDRVTITCRASQDISKYLNWYQQKPGKAPKLLIYHTSRLHSGVPSRFSGSGSGTDYTLTISSLQPEDIATYYCQQANTLPYTFGGGTKLEIK

SEQ ID NO: 37 - protein, 49 aa, Artificial Sequence
  CD8 hinge region
KPTTTPAPRPPTPAPTIASQPLSLRPEASRPAAGGAVHTRGLDFASDKP

SEQ ID NO: 38 - protein, 47 aa, Artificial Sequence
  CD8 hinge region
SGTTTPAPRPPTPAPTIASQPLSLRPEACRPAAGGAVHTRGLDFACD

SEQ ID NO: 39 - protein, 113 aa, Artificial Sequence
  CD3z signaling region
RVKFSRSADAPAYQQGQNQLYNELNLGRREEYDVLDKRRGRDPEMGGKPQRRKNPQEGLYNELQKDKMAEAYSEIGMKGERRRGKGHDGLYQGLSTATKDTYDALHMQALPPR